European Patent Specification EP 3 582 619 B1, published December 25, 2024. Title: LIPOLYTIC ENZYME FOR USE IN BAKING. Applicant: Novozymes A/S Puratos NV. The sequence listing filed with the application follows.

SEQUENCE LISTING (9 sequences)

SEQ ID NO: 1 - protein, 309 aa, Valsaria rubricosa
MKSASILLRVAALLLPAVSALPLERRAISADLLATFSLFEQFAAAAYCPDNNDSPDTKLTCSVGNCPLVEADTTSTVTEFENSLETDVTGYVATDSTRELIVVAFRGSSSIRNWIADIDFPFTDTDLCDGCQAASGFWTSWTEARTGVLAAVASAAAANPSYTVAVTGHSLGGAVAALAAGALRNAGYTVALYSFGAPRVGDETLSEYITAQAGGNYRITHLNDPVPKLPPLLLGYRHISPEYYISSGNNVTVTADDVEEYTGTINLSGNTGDLTFDTDAHSWYFNEIGACDDGEALEWKKRGVEVQWV

SEQ ID NO: 2 - DNA, 1059 bp, Valsaria rubricosa
atgaagtccgcttcgatcttactcagggtagctgccctcctcctccctgctgtatctgcactgccacttgaaagaagaggtatggacgaactatcctagcgatcagtgtgtctattttgcctaacctagcaaagctatatccgcggatctcctggcaaccttcagcctcttcgagcagttcgcagccgcagcatattgtccggataacaacgacagtcccgacaccaagcttacttgctctgtcggaaactgcccgcttgtcgaagctgacacgaccagcacggtcactgaattcgaaaagtacatcttacacgaccccgttcacctacagacaaagtcccagctaacgtccacctctatctctgtccctttagctcgctcgaaaccgacgtcactggctacgtcgcgactgacagcacacgagagctcatcgttgtggcattccgcgggagttcctcgatccggaactggatcgccgacatcgactttcccttcaccgacaccgacctctgcgatggctgccaggcagcctcgggcttctggacgtcctggacggaggcacggacaggggtgctggcggcggtggcgagcgctgccgcggccaacccgtcctataccgttgccgtgacgggccacagcctcggcggggccgtggccgcgctggccgctggcgccctccggaacgcgggctacacggtcgcgctatacagcttcggagcgcctcgcgtgggtgacgagaccctcagcgagtacatcactgcgcaggcgggtggaaactaccgcatcacgcacctcaacgacccagtgccgaagctgcccccgctgctcctggggtatcgccacatcagcccggaatactacatcagcagcgggaacaacgtgaccgtgacggcggatgacgtggaggagtacaccggcacgatcaacctgagtgggaacacgggcgatctgacgttcgacacggatgcgcacagttggtacttcaacgagatcggggcatgcgatgatggtgaggctttggagtggaagaagcggggggtagaagttcagtgggtttaa

SEQ ID NO: 3 - DNA, 46 bp, Artificial Sequence
  Primer
acacaactggggatccaccatgaagtccgcttcgatcttactcagg

SEQ ID NO: 4 - DNA, 40 bp, Artificial Sequence
  Primer
agatctcgagaagcttaaacccactgaacttctacccccc

SEQ ID NO: 5 - protein, 5 aa, Artificial Sequence
  Catalytic segment
GHSLG

SEQ ID NO: 6 - protein, 309 aa, Artificial Sequence
  artificial sequence
MKSASILLRVAALLLPAVSALPLERRAISADLLATFSLFEQFAAAAYCPNNNNSPDTKLTCSQGNCPLVEAATTSTVTEFENSLSTDVTGYVAVDSTRELIVVAFRGSSSIRNWIADIDFPFTDTDLCDGCQAASGFWQSWTEARTGVTAAVASAAAQNPSYTVVVTGHSLGGAVAALAAGALRNQGYTVALYSFGAPRVGNETLSEYITAQAGGNYRITHLNDPVPKLPPLLLGYRHISPEYYISSGNNVTVTANDVEEYTGTINLSGNTGDLTFDTDAHSWYFNEIGACDDGEALEWKKRGVEVQWV

SEQ ID NO: 7 - protein, 309 aa, Artificial Sequence
  artificial sequence
MKSASILLRVAALLLPAVSALPLERRAISADLLATFSLFEQFAAAAYCPNNNNSPGTKLTCSQGNCPLVEAATTNTVTEFENSLSTDVTGYVAVDSTNELIVVSFRGSSSIRNWIADIDFPFTDTDLCDGCQAASGFWQSWTEARTTVTAAVAQAAAQNPSYQVVVTGHSLGGAIAALAAGALRNQGYTVDLYSFGAPRVGNETLSEYITNQAGGNYRITHLNDPVPKLPPLLMGYRHISPEYYISSGNNVTVTANDVQEYTGTINLQGNTGDLTFDIDAHSWYFNEIGACDDGEALEWKKRGVEVQWV

SEQ ID NO: 8 - protein, 309 aa, Artificial Sequence
  artificial sequence
MKSASILLRVAALLLPAVSALPLERRAISADLLATFQFFEQYAAAAYCPNNNNSPGTKLTCSQGNCPLVQAATTNTVYEFENSLSTDVTGYVAVDSTNKLIVVSFRGSSSIRNWIADIDFPFTDTDLCDGCQAASGFWQSWLEARTTVTPAVAQARAQNPDYQVVVTGHSLGGAIAALAAGDLRNQGYTVDLYTFGAPRVGNETLSEYITNQAGGNYRITHWNDPVPKLPPLLMGYVHISPEYYISSGNNVTVTANDVQEYTGTINLQGNTGDLTFDIDAHSWYFNEIGACDDGEALEWKKRGVEVQWV

SEQ ID NO: 9 - protein, 309 aa, Artificial Sequence
  artificial sequence
MKSASILLRVAALLLPAVSALPLERRAISADLLDTFQFFEQYAAAAYCPNNNNSPGTKLTCSQGNCPLVQAADTNTVYEFENSLSTDVTGYVAVDHTNKLIVVSFRGSSSIRNWIADIDFPFTDTDLCDGCQAASGFWQSWLEARDTVTPAVYQARAQKPDYQVVVTGHSLGGAIAALAAGDLRNQGYTVDLYTFGAPRVGNSTLSEYITNQPGGNYRVTHWNDPVPKLPPLLMGYVHISPEYYISSPNNVTVTANDVQVYEGVINLQGNEGDLTTDIDAHSWYFNEIGACDDGEALEWKKRGVEVQWV